European Patent Specification EP 4 180 523 B1, published August 21, 2024. Title: Novel glutamine-hydrolyzing GMP synthase variant and a method for producing purine nucleotide using the same. Applicant: CJ CheilJedang Corporation. The sequence listing filed with the application follows.

SEQUENCE LISTING (51 sequences)

SEQ ID NO: 1 - protein, 524 aa, Artificial Sequence
  guaA_R29C
MTQPATTPRPVLVVDFGAQYAQLIARRVCEASIYSEVVPHSATVKEIKAKNPAALILSGGPSSVYADGAPQLKPELLELGVPVFGICYGFQAMNHALGGNVAQTGDREYGRTEITHTGGVLHDGLEENHKVWMSHGDAVDKAPEGFTVTASSAGAPVAAMECVAKQMAGVQYHPEVMHSPHGQEVLVRFLTEVAGLEQTWTSANIAQQLIDDVRAQIGPEGRAICGLSGGVDSAVAAALVQRAIGDRLTCVFVDHGLLRAGEREQVEKDFVASTGAKLITAHEADAFLSKLAGVTDPEAKRKAIGAEFIRSFERAVAQALEESPEDSTVDFLVQGTLYPDVVESGGGDGTANIKSHHNVGGLPDDVEFELVEPLRLLFKDEVRAVGRELGLPEEIVARQPFPGPGLGIRIIGEVTEERLEILRQADLIARTELTNAGLDGDIWQCPVVLLADVRSVGVQGDGRTYGHPIVLRPVSSEDAMTADWTRVPYDVLEKISTRITNEVNDVNRVVVDITSKPPGTIEWE

SEQ ID NO: 2 - DNA, 1575 bp, Artificial Sequence
  guaA_c85t
gtgactcaacctgcaacaactccgcgcccagtcctcgtggtggatttcggtgcccaatacgcacagctgattgctcgtcgcgtatgtgaggcatcgatttactccgaggtagtcccacattccgccaccgttaaagagattaaagctaaaaaccctgcagctttgattttgtccggtggcccgtcctctgtttatgccgatggcgccccgcaattaaagcctgaactgctcgagcttggtgtgccagtctttggcatctgctacggcttccaagccatgaaccatgctttgggtggcaacgttgcgcaaaccggtgaccgtgaatacggccgcaccgaaatcacccataccggtggtgtgctgcacgacggcttagaagaaaaccacaaggtctggatgtcccacggtgatgctgtggataaggcacctgagggctttaccgtgaccgcatcgtcggctggtgcgccggttgcagcgatggaatgcgtggccaagcaaatggctggtgtgcaataccaccccgaggttatgcattccccacacggacaggaagtactcgttcgcttcctcaccgaggtagcagggctagagcagacctggacctcggcaaatattgcgcagcagcttatcgatgatgtccgcgcgcaaatcggccctgaaggccgcgctatttgtggcctgtcgggcggcgtggactccgcagtcgctgcagcgctcgtgcagcgcgccattggcgaccgtttgacctgtgtgttcgtggaccacggtctgctgcgcgccggtgagcgtgagcaggtagaaaaggacttcgtggcttcgactggtgcgaagctgattaccgcgcatgaagctgatgctttcttgtctaagctcgccggtgttaccgatcctgaggctaagcgcaaggctatcggcgcggaattcatccgttcctttgagcgtgctgtggcacaggctttggaagaatctcctgaagactccacagtggacttcctggtccagggcaccttgtatccggatgtggttgaatccggcggcggtgacggcaccgcaaatatcaagtcccaccacaatgttggcggcctgccagacgatgtcgaattcgaactcgtcgagccactacgcctgctgtttaaggacgaagtccgtgccgtcggccgcgagctcggcctgcctgaggaaatcgttgcccgccagccattccctggccctggcctaggcatccgcatcatcggtgaagtcaccgaggagcgtctagaaatcctgcgtcaagcagacctgattgcgcgtaccgagctgaccaacgctggcctcgacggtgatatctggcagtgcccagtcgtactgcttgccgatgtccgctccgtcggagtccaaggcgacggccgcacctacggccacccaatcgtgctgcgcccagtgtcatccgaggatgccatgaccgccgactggacccgcgttccttacgacgtcctagagaaaatctccacccgcattaccaacgaagtcaacgacgtcaaccgcgtggtcgtcgacatcacctccaagccaccgggaaccatcgagtgggagtaa

SEQ ID NO: 3 - protein, 524 aa, Unknown
  Corynebacterium stationis
MTQPATTPRPVLVVDFGAQYAQLIARRVREASIYSEVVPHSATVKEIKAKNPAALILSGGPSSVYADGAPQLKPELLELGVPVFGICYGFQAMNHALGGNVAQTGDREYGRTEITHTGGVLHDGLEENHKVWMSHGDAVDKAPEGFTVTASSAGAPVAAMECVAKQMAGVQYHPEVMHSPHGQEVLVRFLTEVAGLEQTWTSANIAQQLIDDVRAQIGPEGRAICGLSGGVDSAVAAALVQRAIGDRLTCVFVDHGLLRAGEREQVEKDFVASTGAKLITAHEADAFLSKLAGVTDPEAKRKAIGAEFIRSFERAVAQALEESPEDSTVDFLVQGTLYPDVVESGGGDGTANIKSHHNVGGLPDDVEFELVEPLRLLFKDEVRAVGRELGLPEEIVARQPFPGPGLGIRIIGEVTEERLEILRQADLIARTELTNAGLDGDIWQCPVVLLADVRSVGVQGDGRTYGHPIVLRPVSSEDAMTADWTRVPYDVLEKISTRITNEVNDVNRVVVDITSKPPGTIEWE

SEQ ID NO: 4 - DNA, 1575 bp, Unknown
  Corynebacterium stationis
gtgactcaacctgcaacaactccgcgcccagtcctcgtggtggatttcggtgcccaatacgcacagctgattgctcgtcgcgtacgtgaggcatcgatttactccgaggtagtcccacattccgccaccgttaaagagattaaagctaaaaaccctgcagctttgattttgtccggtggcccgtcctctgtttatgccgatggcgccccgcaattaaagcctgaactgctcgagcttggtgtgccagtctttggcatctgctacggcttccaagccatgaaccatgctttgggtggcaacgttgcgcaaaccggtgaccgtgaatacggccgcaccgaaatcacccataccggtggtgtgctgcacgacggcttagaagaaaaccacaaggtctggatgtcccacggtgatgctgtggataaggcacctgagggctttaccgtgaccgcatcgtcggctggtgcgccggttgcagcgatggaatgcgtggccaagcaaatggctggtgtgcaataccaccccgaggttatgcattccccacacggacaggaagtactcgttcgcttcctcaccgaggtagcagggctagagcagacctggacctcggcaaatattgcgcagcagcttatcgatgatgtccgcgcgcaaatcggccctgaaggccgcgctatttgtggcctgtcgggcggcgtggactccgcagtcgctgcagcgctcgtgcagcgcgccattggcgaccgtttgacctgtgtgttcgtggaccacggtctgctgcgcgccggtgagcgtgagcaggtagaaaaggacttcgtggcttcgactggtgcgaagctgattaccgcgcatgaagctgatgctttcttgtctaagctcgccggtgttaccgatcctgaggctaagcgcaaggctatcggcgcggaattcatccgttcctttgagcgtgctgtggcacaggctttggaagaatctcctgaagactccacagtggacttcctggtccagggcaccttgtatccggatgtggttgaatccggcggcggtgacggcaccgcaaatatcaagtcccaccacaatgttggcggcctgccagacgatgtcgaattcgaactcgtcgagccactacgcctgctgtttaaggacgaagtccgtgccgtcggccgcgagctcggcctgcctgaggaaatcgttgcccgccagccattccctggccctggcctaggcatccgcatcatcggtgaagtcaccgaggagcgtctagaaatcctgcgtcaagcagacctgattgcgcgtaccgagctgaccaacgctggcctcgacggtgatatctggcagtgcccagtcgtactgcttgccgatgtccgctccgtcggagtccaaggcgacggccgcacctacggccacccaatcgtgctgcgcccagtgtcatccgaggatgccatgaccgccgactggacccgcgttccttacgacgtcctagagaaaatctccacccgcattaccaacgaagtcaacgacgtcaaccgcgtggtcgtcgacatcacctccaagccaccgggaaccatcgagtgggagtaa

SEQ ID NO: 5 - DNA, 18 bp, Artificial Sequence
  primer
gcgatgtgattgccggtg

SEQ ID NO: 6 - DNA, 18 bp, Artificial Sequence
  primer
gctctaggaagtcagcag

SEQ ID NO: 7 - DNA, 19 bp, Artificial Sequence
  primer
tgcccaatacgcacagctg

SEQ ID NO: 8 - DNA, 16 bp, Artificial Sequence
  primer
ggctggggctttgtcc

SEQ ID NO: 9 - DNA, 18 bp, Artificial Sequence
  primer
ggcttagcaagacctggc

SEQ ID NO: 10 - DNA, 37 bp, Artificial Sequence
  primer
gtgaattcgagctcggtacccgcaccgcagttagccc

SEQ ID NO: 11 - DNA, 33 bp, Artificial Sequence
  primer
taaatcgatgcctcacatacgcgacgagcaatc

SEQ ID NO: 12 - DNA, 33 bp, Artificial Sequence
  primer
gattgctcgtcgcgtatgtgaggcatcgattta

SEQ ID NO: 13 - DNA, 39 bp, Artificial Sequence
  primer
ggtcgactctagaggatcccccgaggtccaggtctgctc

SEQ ID NO: 14 - DNA, 17 bp, Artificial Sequence
  primer
ggaatccgaagcggagc

SEQ ID NO: 15 - DNA, 18 bp, Artificial Sequence
  primer
caggccacaaatagcgcg

SEQ ID NO: 16 - DNA, 33 bp, Artificial Sequence
  primer
taaatcgatgcctcgcctacgcgacgagcaatc

SEQ ID NO: 17 - DNA, 33 bp, Artificial Sequence
  primer
gattgctcgtcgcgtaggcgaggcatcgattta

SEQ ID NO: 18 - DNA, 33 bp, Artificial Sequence
  primer
taaatcgatgcctcgaatacgcgacgagcaatc

SEQ ID NO: 19 - DNA, 33 bp, Artificial Sequence
  primer
gattgctcgtcgcgtattcgaggcatcgattta

SEQ ID NO: 20 - DNA, 33 bp, Artificial Sequence
  primer
taaatcgatgcctcggatacgcgacgagcaatc

SEQ ID NO: 21 - DNA, 33 bp, Artificial Sequence
  primer
gattgctcgtcgcgtatccgaggcatcgattta

SEQ ID NO: 22 - DNA, 33 bp, Artificial Sequence
  primer
taaatcgatgcctcgtatacgcgacgagcaatc

SEQ ID NO: 23 - DNA, 33 bp, Artificial Sequence
  primer
gattgctcgtcgcgtatacgaggcatcgattta

SEQ ID NO: 24 - DNA, 33 bp, Artificial Sequence
  primer
taaatcgatgcctcccatacgcgacgagcaatc

SEQ ID NO: 25 - DNA, 33 bp, Artificial Sequence
  primer
gattgctcgtcgcgtatgggaggcatcgattta

SEQ ID NO: 26 - DNA, 33 bp, Artificial Sequence
  primer
taaatcgatgcctcgattacgcgacgagcaatc

SEQ ID NO: 27 - DNA, 33 bp, Artificial Sequence
  primer
gattgctcgtcgcgtaatcgaggcatcgattta

SEQ ID NO: 28 - DNA, 33 bp, Artificial Sequence
  primer
taaatcgatgcctccactacgcgacgagcaatc

SEQ ID NO: 29 - DNA, 33 bp, Artificial Sequence
  primer
gattgctcgtcgcgtagtggaggcatcgattta

SEQ ID NO: 30 - DNA, 33 bp, Artificial Sequence
  primer
taaatcgatgcctctggtacgcgacgagcaatc

SEQ ID NO: 31 - DNA, 33 bp, Artificial Sequence
  primer
gattgctcgtcgcgtaccagaggcatcgattta

SEQ ID NO: 32 - DNA, 33 bp, Artificial Sequence
  primer
taaatcgatgcctcggttacgcgacgagcaatc

SEQ ID NO: 33 - DNA, 33 bp, Artificial Sequence
  primer
gattgctcgtcgcgtaaccgaggcatcgattta

SEQ ID NO: 34 - DNA, 33 bp, Artificial Sequence
  primer
taaatcgatgcctctgctacgcgacgagcaatc

SEQ ID NO: 35 - DNA, 33 bp, Artificial Sequence
  primer
gattgctcgtcgcgtagcagaggcatcgattta

SEQ ID NO: 36 - DNA, 33 bp, Artificial Sequence
  primer
taaatcgatgcctcatctacgcgacgagcaatc

SEQ ID NO: 37 - DNA, 33 bp, Artificial Sequence
  primer
gattgctcgtcgcgtagatgaggcatcgattta

SEQ ID NO: 38 - DNA, 33 bp, Artificial Sequence
  primer
taaatcgatgcctcgtttacgcgacgagcaatc

SEQ ID NO: 39 - DNA, 33 bp, Artificial Sequence
  primer
gattgctcgtcgcgtaaacgaggcatcgattta

SEQ ID NO: 40 - DNA, 33 bp, Artificial Sequence
  primer
taaatcgatgcctcgtgtacgcgacgagcaatc

SEQ ID NO: 41 - DNA, 33 bp, Artificial Sequence
  primer
gattgctcgtcgcgtacacgaggcatcgattta

SEQ ID NO: 42 - DNA, 33 bp, Artificial Sequence
  primer
taaatcgatgcctccagtacgcgacgagcaatc

SEQ ID NO: 43 - DNA, 33 bp, Artificial Sequence
  primer
gattgctcgtcgcgtactggaggcatcgattta

SEQ ID NO: 44 - DNA, 33 bp, Artificial Sequence
  primer
taaatcgatgcctccattacgcgacgagcaatc

SEQ ID NO: 45 - DNA, 33 bp, Artificial Sequence
  primer
gattgctcgtcgcgtaatggaggcatcgattta

SEQ ID NO: 46 - DNA, 33 bp, Artificial Sequence
  primer
taaatcgatgcctcctgtacgcgacgagcaatc

SEQ ID NO: 47 - DNA, 33 bp, Artificial Sequence
  primer
gattgctcgtcgcgtacaggaggcatcgattta

SEQ ID NO: 48 - DNA, 33 bp, Artificial Sequence
  primer
taaatcgatgcctcctttacgcgacgagcaatc

SEQ ID NO: 49 - DNA, 33 bp, Artificial Sequence
  primer
gattgctcgtcgcgtaaaggaggcatcgattta

SEQ ID NO: 50 - DNA, 33 bp, Artificial Sequence
  primer
taaatcgatgcctcttctacgcgacgagcaatc

SEQ ID NO: 51 - DNA, 33 bp, Artificial Sequence
  primer
gattgctcgtcgcgtagaagaggcatcgattta